European Patent Application EP 4 768 577 A1, published July 1, 2026. Title: 莱鲍迪苷M的制备方法和β-1,2-葡萄糖基转移酶在其中的应用. Applicant: 弈柯莱生物科技（集团）股份有限公司. The sequence listing filed with the application follows.

SEQUENCE LISTING (24 sequences)

SEQ ID NO: 1 - DNA, 2415 bp, synthetic construct
  source 1..2415: mol_type = other DNA
atgtccgaacgtgcgcgtagcgatgatctgattgaacagctgcgcggcttcctggatgcttgtccgtccgtgggtcatcgcgttctgcaccagattaaaaaactggaacgctccttccttcagcgttctgaactgtgcgacgcgtttgcagatgtttgcgcagccgaagatgttccagatggcctgcgccagagcccgctgggtaaagttattcgtctgacccaggaagccgctgttaacgatgcttgggtttacctggctgttcgtgtgcgtattgcgtcctggcgttacgttcgtatcgcgctggaaggtatggcggttgaagaagtgactgttcgtgatttcctgcgtttcaaagaatgtctggctttgggccagcacgattttgatgaatggctgctggaaattgatctgggtccgttctctcgtgaatttccgaaactgctggaagcccgttccattggccgtggtgttgaatttctgaacaaacatctgagcctgcaactgttcgacgaactgggtgaaggtggtgaacgcatcctgaacttcctgcgcatccactcttttcgcggccagaccctgatgctgaacgaacagattaaatccgtgtctgatctccgtcgtgcactgcgtcgtgcggatgaagtgttggccggtcacgagccgacggcgacctgggaagatgtggctgcaccgctgcgcgcactgggtttcgaagttggttggggtcgtgaagttgcgcgtatccgtgacaccatgagcctgctgcgtgatctgctggaagcaccagaccctcgtggcctggaaacctttctggctcgtctgccgatggtgttttctctggctatcatttctccgcacggttacttcggtcaggctaacgttctgggtcgtccggatactggtggtcaggtggtatacattctggaccaggttcgtgccctcgaaaccgagatgcgctctcgcctgttcgaacagggcctggacatcgaaccgcagattgttgtcctgacccgtctgatcccgcaggctgaaggcaccacctgcgatcagcgtctggaaccgatctctggcactcgcaacgcgcgcatcctgcgtgtcccgttccgtaacgccagcggtgaaatcgttacccactggatttctcgtttcgaggtgtggccttacctggaacgttacactctggatagcgaacgtgaactgctggctgaactgggtggccgtccggatctgatcgttggtaattatagcgacggtaacctggtggctaccctgctgtcccagcgcctgggcgtgacccagtgcaacatcgcacacgcgctggaaaaaaccaaataccctcacgccgacctgttctggcaggaaaacgaagcgcagtatcattttagctgccagtttaccgcggatctgattgctatgaacgctgctgactttatcatcacgtctacctaccaggaaatcgctggtacgcgcgaatccgttggccagtatgagagccacaccgcgttcaccatgccgaaactgttccgtgtggtcaacggcattgacgtgtatgacccaaaattcaacatcgtgagtccgggcgccgacgcagctgcatacttcccgtataccgcggtggaacgtcgcctcccgcatctgcacactgaaatcgaacagctggttttcggcgtggatgaacgtgttgacgcgcgcggcgtgctgaccgaacgtgacaaaccgctgctgttcactatggctcgtttggaccgtatcaaaaacatcgttggtctggttgaatggttcggcgcgtgcgaagcgctgcgtaaagaagcgaatctgctggtcatctcaggtcacgtagacccggaacgctcatccgacactgaagaactggaacagatccgttgtatgcacgctctgttcaaccgttatgatctggatcgtcaggtgcgctggctgggtctgcgtctgccgaaagatctggcgggtgaattttaccgctatgttgcggacggtcgtggcgcgttcgttcagccggctctgtttgaagcattcggtctgaccgtgattgaagcgatggcgtctggcctgccgtgcttcgcaacctgcttcggcggcccgtctgaaatcattgaagatggtgtctctggcttccacatcgatccgaaccacggcgatgcggcagcggaacgtatcgcgcgctttttcgaacgtacccgtcaagatccggaatattggaaccgtatctctgaaggcgcgctgaaacgtgtggccgaacgctacacctggcagcattatgctgaacgtatgatgaccctgagccgtgtttacggcttctggcgtcatgttactgacctggaacgtcgtgaaacccagcgttacctgcaagctctgtattctctgcaattccgtcgtctggcgcaggcgatggcg

SEQ ID NO: 2 - protein, 805 aa, synthetic construct
MSERARSDDLIEQLRGFLDACPSVGHRVLHQIKKLERSFLQRSELCDAFADVCAAEDVPDGLRQSPLGKVIRLTQEAAVNDAWVYLAVRVRIASWRYVRIALEGMAVEEVTVRDFLRFKECLALGQHDFDEWLLEIDLGPFSREFPKLLEARSIGRGVEFLNKHLSLQLFDELGEGGERILNFLRIHSFRGQTLMLNEQIKSVSDLRRALRRADEVLAGHEPTATWEDVAAPLRALGFEVGWGREVARIRDTMSLLRDLLEAPDPRGLETFLARLPMVFSLAIISPHGYFGQANVLGRPDTGGQVVYILDQVRALETEMRSRLFEQGLDIEPQIVVLTRLIPQAEGTTCDQRLEPISGTRNARILRVPFRNASGEIVTHWISRFEVWPYLERYTLDSERELLAELGGRPDLIVGNYSDGNLVATLLSQRLGVTQCNIAHALEKTKYPHADLFWQENEAQYHFSCQFTADLIAMNAADFIITSTYQEIAGTRESVGQYESHTAFTMPKLFRVVNGIDVYDPKFNIVSPGADAAAYFPYTAVERRLPHLHTEIEQLVFGVDERVDARGVLTERDKPLLFTMARLDRIKNIVGLVEWFGACEALRKEANLLVISGHVDPERSSDTEELEQIRCMHALFNRYDLDRQVRWLGLRLPKDLAGEFYRYVADGRGAFVQPALFEAFGLTVIEAMASGLPCFATCFGGPSEIIEDGVSGFHIDPNHGDAAAERIARFFERTRQDPEYWNRISEGALKRVAERYTWQHYAERMMTLSRVYGFWRHVTDLERRETQRYLQALYSLQFRRLAQAMA

SEQ ID NO: 3 - DNA, 1350 bp, synthetic construct
  source 1..1350: mol_type = other DNA
atgcaccatcatcatgaaggcgtgagcgaccagaccctgagagtaacgatgtttccgtggcttgggctgggtcatgttaacccgtttttgcgtatcgctaaacaactggccgatcgtggtttcgttatctatttagttagtaccgctattaacctcgaaatgatcaaaaagagaatcccggagaaatacagtaatagcatccatctggttgagctgcgcctgccagaattaccggaactgccaccacattaccatactaccaacggtttaccaccgcatctgaacaaaaccctgcacaaggcactgaagatgagcgctcccaactttagcaagatccttcaaaatattaagccggacctggtcctttacgattttctggttccgtgggcagaaaaagtcgcgcttgaacagggcatcccggctgttccattgctaaccagtggtgcggcactgttcagctactttttcaacttcctgaagcgaccgggtgaagagtttccgtttgaggcaatccgcctgtcgaagcgagaacaggataagatgcgcgagatgtttggaacagagccgcctgaagaagattttttagcgccggcccaggccggtatcatgctgatgtgcacgagccgcgtaattgaggctaagtacctggactattgtaccgaactgaccaatgtaaaagttgttccggttggtccgccgtttcaggatccgctgaccgaagatattgacgaccccgaactgatggattggttagataccaaacccgaacatagtgttgtctatgtgtcgtttggcagcgaagcgttcctgagccgtgaagatatggaagaagtcgcgttcggcctggagctgagcggcgtgaactttatctgggttgcacgctttccgaaaggcgaagaacagcgtctggaagacgttctgccaaaaggcttcctggaacgcgttggtgatcgtggtcgcgttctggaccatctggtgccgcaggcccatattctgaaccatccgagcacgggtggcttcatctctcattgcggttggaacagcgtcatggaaagcattgatttcggcgttccgatcattgcgatgccgatgcagtgggatcagccgattaacgcgagactgcttgtggaattaggcgtggcagtggagatcccgcgtgatgaagatggccgggtccaccgcgccgaaattgccgaagcactgaaaagcgttgtgaccggtgaaaccggcgaaatcctgcgtgcgaaagttcgtgaaatcagcaaaaacctgaaatccatccgtgacgaagaaatggacgcggttgctgaagaactgatccagctgtgccgtaactctaacaaaagcaaa

SEQ ID NO: 4 - protein, 450 aa, synthetic construct
MHHHHEGVSDQTLRVTMFPWLGLGHVNPFLRIAKQLADRGFVIYLVSTAINLEMIKKRIPEKYSNSIHLVELRLPELPELPPHYHTTNGLPPHLNKTLHKALKMSAPNFSKILQNIKPDLVLYDFLVPWAEKVALEQGIPAVPLLTSGAALFSYFFNFLKRPGEEFPFEAIRLSKREQDKMREMFGTEPPEEDFLAPAQAGIMLMCTSRVIEAKYLDYCTELTNVKVVPVGPPFQDPLTEDIDDPELMDWLDTKPEHSVVYVSFGSEAFLSREDMEEVAFGLELSGVNFIWVARFPKGEEQRLEDVLPKGFLERVGDRGRVLDHLVPQAHILNHPSTGGFISHCGWNSVMESIDFGVPIIAMPMQWDQPINARLLVELGVAVEIPRDEDGRVHRAEIAEALKSVVTGETGEILRAKVREISKNLKSIRDEEMDAVAEELIQLCRNSNKSK

SEQ ID NO: 5 - DNA, 33 bp, synthetic construct
  source 1..33: mol_type = other DNA
gtcgcgttctgaacaaactggtgccgcaggccc

SEQ ID NO: 6 - DNA, 33 bp, synthetic construct
  source 1..33: mol_type = other DNA
ggcaccagtttgttcagaacgcgaccacgatca

SEQ ID NO: 7 - DNA, 40 bp, synthetic construct
  source 1..40: mol_type = other DNA
cgcgagatgttgggaacatttccgcctgaagaagattttt

SEQ ID NO: 8 - DNA, 41 bp, synthetic construct
  source 1..41: mol_type = other DNA
tgttcccaacatctcgcgcaacttatcctgttctcgcttcg

SEQ ID NO: 9 - DNA, 35 bp, synthetic construct
  source 1..35: mol_type = other DNA
ttccgtttcaggcccctatcatgctgatgtgcacg

SEQ ID NO: 10 - DNA, 40 bp, synthetic construct
  source 1..40: mol_type = other DNA
taggggcctgaaacggaactaaaaaatcttcttcaggcgg

SEQ ID NO: 11 - DNA, 31 bp, synthetic construct
  source 1..31: mol_type = other DNA
gcgaaactgatggtggaattaggcgtggcag

SEQ ID NO: 12 - DNA, 34 bp, synthetic construct
  source 1..34: mol_type = other DNA
attccaccatcagtttcgcgttaatcggctgatc

SEQ ID NO: 13 - DNA, 31 bp, synthetic construct
  source 1..31: mol_type = other DNA
gaacaaattcgcgccgcaggcccatattctg

SEQ ID NO: 14 - DNA, 30 bp, synthetic construct
  source 1..30: mol_type = other DNA
ctgcggcgcgaatttgttcagaacgcgacc

SEQ ID NO: 15 - DNA, 1350 bp, synthetic construct
  source 1..1350: mol_type = other DNA
atgcaccatcatcatgaaggcgtgagcgaccagaccctgagagtaacgatgtttccgtggcttgggctgggtcatgttaacccgtttttgcgtatcgctaaacaactggccgatcgtggtttcgttatctatttagttagtaccgctattaacctcgaaatgatcaaaaagagaatcccggagaaatacagtaatagcatccatctggttgagctgcgcctgccagaattaccggaactgccaccacattaccatactaccaacggtttaccaccgcatctgaacaaaaccctgcacaaggcactgaagatgagcgctcccaactttagcaagatccttcaaaatattaagccggacctggtcctttacgattttctggttccgtgggcagaaaaagtcgcgcttgaacagggcatcccggctgttccattgctaaccagtggtgcggcactgttcagctactttttcaacttcctgaagcgaccgggtgaagagtttccgtttgaggcaatccgcctgtcgaagcgagaacaggataagttgcgcgagatgttgggaacatttccgcctgaagaagattttttagcgccggcccaggccggtatcatgctgatgtgcacgagccgcgtaattgaggctaagtacctggactattgtaccgaactgaccaatgtaaaagttgttccggttggtccgccgtttcaggatccgctgaccgaagatattgacgaccccgaactgatggattggttagataccaaacccgaacatagtgttgtctatgtgtcgtttggcagcgaagcgttcctgagccgtgaagatatggaagaagtcgcgttcggcctggagctgagcggcgtgaactttatctgggttgcacgctttccgaaaggcgaagaacagcgtctggaagacgttctgccaaaaggcttcctggaacgcgttggtgatcgtggtcgcgttctgaacaaactggtgccgcaggcccatattctgaaccatccgagcacgggtggcttcatctctcattgcggttggaacagcgtcatggaaagcattgatttcggcgttccgatcattgcgatgccgatgcagtgggatcagccgattaacgcgagactgcttgtggaattaggcgtggcagtggagatcccgcgtgatgaagatggccgggtccaccgcgccgaaattgccgaagcactgaaaagcgttgtgaccggtgaaaccggcgaaatcctgcgtgcgaaagttcgtgaaatcagcaaaaacctgaaatccatccgtgacgaagaaatggacgcggttgctgaagaactgatccagctgtgccgtaactctaacaaaagcaaa

SEQ ID NO: 16 - protein, 450 aa, synthetic construct
MHHHHEGVSDQTLRVTMFPWLGLGHVNPFLRIAKQLADRGFVIYLVSTAINLEMIKKRIPEKYSNSIHLVELRLPELPELPPHYHTTNGLPPHLNKTLHKALKMSAPNFSKILQNIKPDLVLYDFLVPWAEKVALEQGIPAVPLLTSGAALFSYFFNFLKRPGEEFPFEAIRLSKREQDKLREMLGTFPPEEDFLAPAQAGIMLMCTSRVIEAKYLDYCTELTNVKVVPVGPPFQDPLTEDIDDPELMDWLDTKPEHSVVYVSFGSEAFLSREDMEEVAFGLELSGVNFIWVARFPKGEEQRLEDVLPKGFLERVGDRGRVLNKLVPQAHILNHPSTGGFISHCGWNSVMESIDFGVPIIAMPMQWDQPINARLLVELGVAVEIPRDEDGRVHRAEIAEALKSVVTGETGEILRAKVREISKNLKSIRDEEMDAVAEELIQLCRNSNKSK

SEQ ID NO: 17 - DNA, 1350 bp, synthetic construct
  source 1..1350: mol_type = other DNA
atgcaccatcatcatgaaggcgtgagcgaccagaccctgagagtaacgatgtttccgtggcttgggctgggtcatgttaacccgtttttgcgtatcgctaaacaactggccgatcgtggtttcgttatctatttagttagtaccgctattaacctcgaaatgatcaaaaagagaatcccggagaaatacagtaatagcatccatctggttgagctgcgcctgccagaattaccggaactgccaccacattaccatactaccaacggtttaccaccgcatctgaacaaaaccctgcacaaggcactgaagatgagcgctcccaactttagcaagatccttcaaaatattaagccggacctggtcctttacgattttctggttccgtgggcagaaaaagtcgcgcttgaacagggcatcccggctgttccattgctaaccagtggtgcggcactgttcagctactttttcaacttcctgaagcgaccgggtgaagagtttccgtttgaggcaatccgcctgtcgaagcgagaacaggataagatgcgcgagatgtttggaacagagccgcctgaagaagattttttagttccgtttcaggcccctatcatgctgatgtgcacgagccgcgtaattgaggctaagtacctggactattgtaccgaactgaccaatgtaaaagttgttccggttggtccgccgtttcaggatccgctgaccgaagatattgacgaccccgaactgatggattggttagataccaaacccgaacatagtgttgtctatgtgtcgtttggcagcgaagcgttcctgagccgtgaagatatggaagaagtcgcgttcggcctggagctgagcggcgtgaactttatctgggttgcacgctttccgaaaggcgaagaacagcgtctggaagacgttctgccaaaaggcttcctggaacgcgttggtgatcgtggtcgcgttctgaacaaactggtgccgcaggcccatattctgaaccatccgagcacgggtggcttcatctctcattgcggttggaacagcgtcatggaaagcattgatttcggcgttccgatcattgcgatgccgatgcagtgggatcagccgattaacgcgagactgcttgtggaattaggcgtggcagtggagatcccgcgtgatgaagatggccgggtccaccgcgccgaaattgccgaagcactgaaaagcgttgtgaccggtgaaaccggcgaaatcctgcgtgcgaaagttcgtgaaatcagcaaaaacctgaaatccatccgtgacgaagaaatggacgcggttgctgaagaactgatccagctgtgccgtaactctaacaaaagcaaa

SEQ ID NO: 18 - protein, 450 aa, synthetic construct
MHHHHEGVSDQTLRVTMFPWLGLGHVNPFLRIAKQLADRGFVIYLVSTAINLEMIKKRIPEKYSNSIHLVELRLPELPELPPHYHTTNGLPPHLNKTLHKALKMSAPNFSKILQNIKPDLVLYDFLVPWAEKVALEQGIPAVPLLTSGAALFSYFFNFLKRPGEEFPFEAIRLSKREQDKMREMFGTEPPEEDFLVPFQAPIMLMCTSRVIEAKYLDYCTELTNVKVVPVGPPFQDPLTEDIDDPELMDWLDTKPEHSVVYVSFGSEAFLSREDMEEVAFGLELSGVNFIWVARFPKGEEQRLEDVLPKGFLERVGDRGRVLNKLVPQAHILNHPSTGGFISHCGWNSVMESIDFGVPIIAMPMQWDQPINARLLVELGVAVEIPRDEDGRVHRAEIAEALKSVVTGETGEILRAKVREISKNLKSIRDEEMDAVAEELIQLCRNSNKSK

SEQ ID NO: 19 - DNA, 1350 bp, synthetic construct
  source 1..1350: mol_type = other DNA
atgcaccatcatcatgaaggcgtgagcgaccagaccctgagagtaacgatgtttccgtggcttgggctgggtcatgttaacccgtttttgcgtatcgctaaacaactggccgatcgtggtttcgttatctatttagttagtaccgctattaacctcgaaatgatcaaaaagagaatcccggagaaatacagtaatagcatccatctggttgagctgcgcctgccagaattaccggaactgccaccacattaccatactaccaacggtttaccaccgcatctgaacaaaaccctgcacaaggcactgaagatgagcgctcccaactttagcaagatccttcaaaatattaagccggacctggtcctttacgattttctggttccgtgggcagaaaaagtcgcgcttgaacagggcatcccggctgttccattgctaaccagtggtgcggcactgttcagctactttttcaacttcctgaagcgaccgggtgaagagtttccgtttgaggcaatccgcctgtcgaagcgagaacaggataagatgcgcgagatgtttggaacagagccgcctgaagaagattttttagcgccggcccaggccggtatcatgctgatgtgcacgagccgcgtaattgaggctaagtacctggactattgtaccgaactgaccaatgtaaaagttgttccggttggtccgccgtttcaggatccgctgaccgaagatattgacgaccccgaactgatggattggttagataccaaacccgaacatagtgttgtctatgtgtcgtttggcagcgaagcgttcctgagccgtgaagatatggaagaagtcgcgttcggcctggagctgagcggcgtgaactttatctgggttgcacgctttccgaaaggcgaagaacagcgtctggaagacgttctgccaaaaggcttcctggaacgcgttggtgatcgtggtcgcgttctgaacaaactggtgccgcaggcccatattctgaaccatccgagcacgggtggcttcatctctcattgcggttggaacagcgtcatggaaagcattgatttcggcgttccgatcattgcgatgccgatgcagtgggatcagccgattaacgcgaaactgatggtggaattaggcgtggcagtggagatcccgcgtgatgaagatggccgggtccaccgcgccgaaattgccgaagcactgaaaagcgttgtgaccggtgaaaccggcgaaatcctgcgtgcgaaagttcgtgaaatcagcaaaaacctgaaatccatccgtgacgaagaaatggacgcggttgctgaagaactgatccagctgtgccgtaactctaacaaaagcaaa

SEQ ID NO: 20 - protein, 450 aa, synthetic construct
MHHHHEGVSDQTLRVTMFPWLGLGHVNPFLRIAKQLADRGFVIYLVSTAINLEMIKKRIPEKYSNSIHLVELRLPELPELPPHYHTTNGLPPHLNKTLHKALKMSAPNFSKILQNIKPDLVLYDFLVPWAEKVALEQGIPAVPLLTSGAALFSYFFNFLKRPGEEFPFEAIRLSKREQDKMREMFGTEPPEEDFLAPAQAGIMLMCTSRVIEAKYLDYCTELTNVKVVPVGPPFQDPLTEDIDDPELMDWLDTKPEHSVVYVSFGSEAFLSREDMEEVAFGLELSGVNFIWVARFPKGEEQRLEDVLPKGFLERVGDRGRVLNKLVPQAHILNHPSTGGFISHCGWNSVMESIDFGVPIIAMPMQWDQPINAKLMVELGVAVEIPRDEDGRVHRAEIAEALKSVVTGETGEILRAKVREISKNLKSIRDEEMDAVAEELIQLCRNSNKSK

SEQ ID NO: 21 - DNA, 1350 bp, synthetic construct
  source 1..1350: mol_type = other DNA
atgcaccatcatcatgaaggcgtgagcgaccagaccctgagagtaacgatgtttccgtggcttgggctgggtcatgttaacccgtttttgcgtatcgctaaacaactggccgatcgtggtttcgttatctatttagttagtaccgctattaacctcgaaatgatcaaaaagagaatcccggagaaatacagtaatagcatccatctggttgagctgcgcctgccagaattaccggaactgccaccacattaccatactaccaacggtttaccaccgcatctgaacaaaaccctgcacaaggcactgaagatgagcgctcccaactttagcaagatccttcaaaatattaagccggacctggtcctttacgattttctggttccgtgggcagaaaaagtcgcgcttgaacagggcatcccggctgttccattgctaaccagtggtgcggcactgttcagctactttttcaacttcctgaagcgaccgggtgaagagtttccgtttgaggcaatccgcctgtcgaagcgagaacaggataagatgcgcgagatgtttggaacagagccgcctgaagaagattttttagcgccggcccaggccggtatcatgctgatgtgcacgagccgcgtaattgaggctaagtacctggactattgtaccgaactgaccaatgtaaaagttgttccggttggtccgccgtttcaggatccgctgaccgaagatattgacgaccccgaactgatggattggttagataccaaacccgaacatagtgttgtctatgtgtcgtttggcagcgaagcgttcctgagccgtgaagatatggaagaagtcgcgttcggcctggagctgagcggcgtgaactttatctgggttgcacgctttccgaaaggcgaagaacagcgtctggaagacgttctgccaaaaggcttcctggaacgcgttggtgatcgtggtcgcgttctgaacaaattcgcgccgcaggcccatattctgaaccatccgagcacgggtggcttcatctctcattgcggttggaacagcgtcatggaaagcattgatttcggcgttccgatcattgcgatgccgatgcagtgggatcagccgattaacgcgagactgcttgtggaattaggcgtggcagtggagatcccgcgtgatgaagatggccgggtccaccgcgccgaaattgccgaagcactgaaaagcgttgtgaccggtgaaaccggcgaaatcctgcgtgcgaaagttcgtgaaatcagcaaaaacctgaaatccatccgtgacgaagaaatggacgcggttgctgaagaactgatccagctgtgccgtaactctaacaaaagcaaa

SEQ ID NO: 22 - protein, 450 aa, synthetic construct
MHHHHEGVSDQTLRVTMFPWLGLGHVNPFLRIAKQLADRGFVIYLVSTAINLEMIKKRIPEKYSNSIHLVELRLPELPELPPHYHTTNGLPPHLNKTLHKALKMSAPNFSKILQNIKPDLVLYDFLVPWAEKVALEQGIPAVPLLTSGAALFSYFFNFLKRPGEEFPFEAIRLSKREQDKMREMFGTEPPEEDFLAPAQAGIMLMCTSRVIEAKYLDYCTELTNVKVVPVGPPFQDPLTEDIDDPELMDWLDTKPEHSVVYVSFGSEAFLSREDMEEVAFGLELSGVNFIWVARFPKGEEQRLEDVLPKGFLERVGDRGRVLNKFAPQAHILNHPSTGGFISHCGWNSVMESIDFGVPIIAMPMQWDQPINARLLVELGVAVEIPRDEDGRVHRAEIAEALKSVVTGETGEILRAKVREISKNLKSIRDEEMDAVAEELIQLCRNSNKSK

SEQ ID NO: 23 - DNA, 1371 bp, synthetic construct
  source 1..1371: mol_type = other DNA
atgccgaacactaacccaactaccgtgcgtcgtcgtcgtgttattatgtttccggttccgttcccgggccacttaaacccgatgctgcaactggcgaacgtgctgtaccgtagaggttttgaaatcaccattctgcacaccaacttcaacgccccgaaaaccagcctttatccgcacttccagtttcgttttatcttggacaacgatccgcaaccggagtggttacgcaacctgccgacgactggtccgggcgtgggtgcaagaatcccggtaattaacaaacacggcgcggatgaattccgtaaggagctggaaatctgcatgcgggatactccgagtgacgaggaagttgcttgcgtgattaccgatgcgctgtggtacttcgcgcaaccggtggcggacagcctgaatctgaaacgtctggttctgcagaccgggagcctgtttaacttccactgcctggtgtgtctgccgaaatttctggagttgggctacctggatccggaaactaaacatcgtccggatgaaccggtggtaggtttcccgatgctgaaggttaaagatatccgtcgcgcgtattcgcacattcaagaatcgaaaccaattctgatgaagatggttgaagaaacccgtgccagcagcggtgtgatttggaacagcgctaaagagctggaggaaagcgagctggaaaccattcagcgtgaaattccggcgccgagcttcctgcttccgctgccgaagcattatagggcttcgagcactagcctgctggatactgatccgagcaccgcccaatggctggaccagcagccgccgagcagcgtgctgtacgttggctttggcagccagagctcgctggaccccgcagatttcctggagattgcgcgtggtctggttgcgagcaaacaaagctttctgtggaacgttcgtccgggcttcgtgaagggttatgagtggattgagctgctgccggatggttttctgggtgaaaaaggtcgtatcgtgaagtctgctccgcaacaagaagtgctggcgcacaaggcgattggtgcgttctggacccacggcggttggaacggcaccatggaggccgtgtgcgaaggcgtgccgatgatctttagcgatttcggtctggatcagccgctgaacgcgcgttacatgagcgaggttctgcatgtgggcgtttatctggagaacggcttcatccgtggtgagatcattaatgcggttaggcgtgtgatggttgaccctgagggtgaggttatgcgccaaaacgcgcgtaaattgaaggataagttggatcgaagcattgctcccggtggcagcagctacgagagcctggaacgcctggagagctatattagcagcctg

SEQ ID NO: 24 - protein, 456 aa, synthetic construct
MPNTNPTTVRRRRVIMFPVPFPGHLNPMLQLANVLYRRGFEITILHTNFNAPKTSLYPHFQFRFILDNDPQPEWLRNLPTTGPGVGARIPVINKHGADEFRKELEICMRDTPSDEEVACVITDALWYFAQPVADSLNLKRLVLQTGSLFNFHCLVCLPKFLELGYLDPETKHRPDEPVVGFPMLKVKDIRRAYSHIQESKPILMKMVEETRASSGVIWNSAKELEESELETIQREIPAPSFLLPLPKHYRASSTSLLDTDPSTAQWLDQQPPSSVLYVGFGSQSSLDPADFLEIARGLVASKQSFLWNVRPGFVKGYEWIELLPDGFLGEKGRIVKSAPQQEVLAHKAIGAFWTHGGWNGTMEAVCEGVPMIFSDFGLDQPLNARYMSEVLHVGVYLENGFIRGEIINAVRRVMVDPEGEVMRQNARKLKDKLDRSIAPGGSSYESLERLESYISS